European Patent Application EP 4 537 853 A1, published April 16, 2025. Title: ANTI-B7H3 ANTIBODY-DRUG CONJUGATE AND USE THEREOF. Applicant: Duality Biologics (Suzhou) Co., Ltd. Application EP 23819114.2, filed June 6, 2023. The sequence listing filed with the application follows.

SEQUENCE LISTING (18 sequences)

SEQ ID NO: 1 - protein, 11 aa, synthetic construct
DYSITGDYAWN

SEQ ID NO: 2 - protein, 16 aa, synthetic construct
YISYSGSTSYNPSLQS

SEQ ID NO: 3 - protein, 10 aa, synthetic construct
SLGRRWYFVV

SEQ ID NO: 4 - protein, 17 aa, synthetic construct
KSSQSLLQSSNQKNYLA

SEQ ID NO: 5 - protein, 7 aa, synthetic construct
FASTRES

SEQ ID NO: 6 - protein, 9 aa, synthetic construct
QQHYSAPWT

SEQ ID NO: 7 - protein, 17 aa, synthetic construct
KSSQSLLNSSNQKNYLA

SEQ ID NO: 8 - protein, 119 aa, synthetic construct
DVQLQESGPGLVKPSQSLSLTCTVTDYSITGDYAWNWIRQFPGNKLEWMGYISYSGSTSYNPSLQSRISITRDTSKNQFFLQLNSVTSEDTATYFCARSLGRRWYFVVWGAGTTVTVSA

SEQ ID NO: 9 - protein, 113 aa, synthetic construct
DIVMTQSPSSLAMSVGQKVTMSCKSSQSLLNSSNQKNYLAWYQQKPGQSPKLLIYFASTRESGVPDRFIGSGSGTDFTLTISSVQAEDLTDYFCQQHYSAPWTFGGGTKLEIK

SEQ ID NO: 10 - protein, 119 aa, synthetic construct
QVQLQESGPGLVKPSQTLSLTCTVTDYSITGDYAWNWIRQHPGKGLEWIGYISYSGSTSYNPSLQSRVTISRDTSKNQFSLKLSSVTAADTAVYFCARSLGRRWYFVVWGQGTTVTVSS

SEQ ID NO: 11 - protein, 113 aa, synthetic construct
DIVMTQSPDSLAVSLGERATINCKSSQSLLQSSNQKNYLAWYQQKPGQPPKLLIYFASTRESGVPDRFSGSGSGTDFTLTISSLQAEDVAVYYCQQHYSAPWTFGGGTKVEIK

SEQ ID NO: 12 - protein, 449 aa, synthetic construct
QVQLQESGPGLVKPSQTLSLTCTVTDYSITGDYAWNWIRQHPGKGLEWIGYISYSGSTSYNPSLQSRVTISRDTSKNQFSLKLSSVTAADTAVYFCARSLGRRWYFVVWGQGTTVTVSSASTKGPSVFPLAPSSKSTSGGTAALGCLVKDYFPEPVTVSWNSGALTSGVHTFPAVLQSSGLYSLSSVVTVPSSSLGTQTYICNVNHKPSNTKVDKRVEPKSCDKTHTCPPCPAPEAAGGPSVFLFPPKPKDTLMISRTPEVTCVVVDVSHEDPEVKFNWYVDGVEVHNAKTKPREEQYNSTYRVVSVLTVLHQDWLNGKEYKCKVSNKALPAPIEKTISKAKGQPREPQVYTLPPSREEMTKNQVSLTCLVKGFYPSDIAVEWESNGQPENNYKTTPPVLDSDGSFFLYSKLTVDKSRWQQGNVFSCSVMHEALHNHYTQKSLSLSPGK

SEQ ID NO: 13 - protein, 220 aa, synthetic construct
DIVMTQSPDSLAVSLGERATINCKSSQSLLQSSNQKNYLAWYQQKPGQPPKLLIYFASTRESGVPDRFSGSGSGTDFTLTISSLQAEDVAVYYCQQHYSAPWTFGGGTKVEIKRTVAAPSVFIFPPSDEQLKSGTASVVCLLNNFYPREAKVQWKVDNALQSGNSQESVTEQDSKDSTYSLSSTLTLSKADYEKHKVYACEVTHQGLSSPVTKSFNRGEC

SEQ ID NO: 14 - protein, 448 aa, synthetic construct
DVQLQESGPGLVKPSQSLSLTCTVTDYSITGDYAWNWIRQFPGNKLEWMGYISYSGSTSYNPSLQSRISITRDTSKNQFFLQLNSVTSEDTATYFCARSLGRRWYFVVWGAGTTVTVSAASTKGPSVFPLAPSSKSTSGGTAALGCLVKDYFPEPVTVSWNSGALTSGVHTFPAVLQSSGLYSLSSVVTVPSSSLGTQTYICNVNHKPSNTKVDKRVEPKSCDKTHTCPPCPAPEAAGGPSVFLFPPKPKDTLMISRTPEVTCVVVDVSHEDPEVKFNWYVDGVEVHNAKTKPREEQYNSTYRVVSVLTVLHQDWLNGKEYKCKVSNKALPAPIEKTISKAKGQPREPQVYTLPPSREEMTKNQVSLTCLVKGFYPSDIAVEWESNGQPENNYKTTPPVLDSDGSFFLYSKLTVDKSRWQQGNVFSCSVMHEALHNHYTQKSLSLSPG

SEQ ID NO: 15 - protein, 220 aa, synthetic construct
DIVMTQSPSSLAMSVGQKVTMSCKSSQSLLNSSNQKNYLAWYQQKPGQSPKLLIYFASTRESGVPDRFIGSGSGTDFTLTISSVQAEDLTDYFCQQHYSAPWTFGGGTKLEIKRTVAAPSVFIFPPSDEQLKSGTASVVCLLNNFYPREAKVQWKVDNALQSGNSQESVTEQDSKDSTYSLSSTLTLSKADYEKHKVYACEVTHQGLSSPVTKSFNRGEC

SEQ ID NO: 16 - protein, 119 aa, synthetic construct; identical to SEQ ID NO: 8

SEQ ID NO: 17 - protein, 113 aa, synthetic construct; identical to SEQ ID NO: 9

SEQ ID NO: 18 - protein, 17 aa, synthetic construct
KSSQSLLNPSNQKNYLA